European Patent Specification EP 3 323 895 B1, published July 23, 2025. Title: Methods, Compositions And Kits For Extraction And Purification Of Adeno-Associated Virus And Adenovirus From Host Cells. Applicant: He, Dao-Yao. The sequence listing filed with the application follows.

SEQUENCE LISTING (6 sequences)

SEQ ID NO: 1 - DNA, 21 bp, Artificial Sequence
  Synthetic
tctgcaccaccggcaagctgc

SEQ ID NO: 2 - DNA, 21 bp, Artificial Sequence
  Synthetic
gagaagcactgcacgccgtag

SEQ ID NO: 3 - DNA, 22 bp, Artificial Sequence
  Synthetic
ggtctccaactcctaatctcag

SEQ ID NO: 4 - DNA, 22 bp, Artificial Sequence
  Synthetic
aaaatcagaaggacagggaagg

SEQ ID NO: 5 - DNA, 24 bp, Artificial Sequence
  Synthetic
ttcctacttggcagtacatctacg

SEQ ID NO: 6 - DNA, 21 bp, Artificial Sequence
  Synthetic
gtcaatggggtggagacttgg